European Patent Application EP 4 435 089 A1, published September 25, 2024. Title: 모든 종류의 필수 아미노산을 포함하는 균사체를 생성하는 아스퍼질러스 오리제 균주. Applicant: CJ CheilJedang Corporation. The sequence listing filed with the application follows.

SEQUENCE LISTING (5 sequences)

SEQ ID NO: 1 - DNA, 1653 bp, synthetic construct
  source 1..1653: mol_type = other DNA
aagcactttatactgtgaactgcgaatggctcattaaatcagttatcgtttatttgatagtaccttactacatggatacctgtggtaattctagagctaatacatgctaaaaacctcgacttcggaaggggtgtatttattagataaaaaaccaatgcccttcggggctccttggtgattcataataacttaacgaatcgcatggccttgcgccggcgatggttcattcaaatttctgccctatcaactttcgatggtaggatagtggcctaccatggtggcaacgggtaacggggaattagggttcgattccggagagggagcctgagaaacggctaccacatccaaggaaggcagcaggcgcgcaaattacccaatcccgacacggggaggtagtgacaataaatactgatacggggctcttttgggtctcgtaattggaatgagtacaatctaaatcccttaacgaggaacaattggagggcaagtctggtgccagcagccgcggtaattccagctccaatagcgtatattaaagttgttgcagttaaaaagctcgtagttgaaccttgggtctggctggccggtccgcctcaccgcgagtactggtccggctggacctttccttctggggaacctcatggccttcactggctgtggggggaaccaggacttttactgtgaaaaaattagagtgttcaaagcaggcctttgctcgaatacattagcatggaataatagaataggacgtgcggttctattttgttggtttctaggaccgccgtaatgattaatagggatagtcgggggcgtcagtattcagctgtcagaggtgaaattcttggatttgctgaagactaactactgcgaaagcattcgccaaggatgttttcattaatcagggaacgaaagttaggggatcgaagacgatcagataccgtcgtagtcttaaccataaactatgccgactagggatcgggcggtgtttctatgatgacccgctcggcaccttacgagaaatcaaagtttttgggttctggggggagtatggtcgcaaggctgaaacttaaagaaattgacggaagggcaccacaaggcgtggagcctgcggcttaatttgactcaacacggggaaactcaccaggtccagacaaaataaggattgacagattgagagctctttcttgatcttttggatggtggtgcatggccgttcttagttggtggagtgatttgtctgcttaattgcgataacgaacgagacctcggcccttaaatagcccggtccgcgtttgcgggccgctggcttcttagggggactatcggctcaagccgatggaagtgcgcggcaataacaggtctgtgatgcccttagatgttctgggccgcacgcgcgctacactgacagggccagcgagtacatcaccttggccgagaggtccgggtaatcttgttaaaccctgtcgtgctggggatagagcattgcaattattgctcttcaacgaggaatgcctagtaggcacgagtcatcagctcgtgccgattacgtccctgccctttgtacacaccgcccgtcgctactaccgattgaatggctcggtgaggccttcggactggcccaggagggttggcaacgaccccccagggccggaa

SEQ ID NO: 2 - DNA, 19 bp, synthetic construct
  source 1..19: mol_type = other DNA
gtagtcatatgcttgtctc

SEQ ID NO: 3 - DNA, 20 bp, synthetic construct
  source 1..20: mol_type = other DNA
tccgcaggttcacctacgga

SEQ ID NO: 4 - DNA, 319 bp, synthetic construct
  source 1..319: mol_type = other DNA
gcccagcctcttggtccaccaaacaacatcaggggaatatccacccttcggcggcccctgagcaaacatcgaaccactgagaaaggtatgcggaaatccaggatcgaactcatatgcattctctattgtgttcacctcttcatccgtcagtgaaatgtgcacagcgggctccacgcccatgagatgctcgactttgcgggctccaacaatgggaaacacatatggggttttctgcaccacatacgccagcgccacttgcaatacggtcaccaccatcaagcacaatcaccatcggctgcgacgaggaatcatcaagtcc

SEQ ID NO: 5 - DNA, 882 bp, synthetic construct
  source 1..882: mol_type = other DNA
acaaaacagtactcaacgcctcatgctcatacccaggcccacactcatgctcattctcatccgcaaccgcatccacaatctcatcctcaatcgaatcaaccaccacacgctctgcccaccccgaatggtagcagtagcgtctccgccatcttttctcatcagagtccgccgccacccgtggagacccagggccttggaggagatctggctggtcaggagcaaagcaccctgtcttccctaacagtcgattcggaattcgggggctcgttgcagtcaatggaacacggaaaccatgccgatttcttggccgagtcgacggggagtcttttcgacgcgtttttggaagtagggacccccatgatcgacccgttcctcgagtcggccccactaccaccgtttcaggcgcgctattgctgcttttcgctagcactacaaacactgacccacctcttcccccacgccccgctgggctgtcaactacggctgacggacggtgaggacagttcgtacaacctgatgacgactgatatggtcatctcggggaacaagagggctaccgatgcggtccggaagatcctcgggtgttcgtgcgcgcaggatggctacttgctgagcatggtcgtccttatcgttctcaaggtgctggcatggtatgctgcggcagcaggcacccagtgtacctcaacggcggcgagtggagaaaccaacagtggcagctgtagcaacagtcccgccaccgtgtccagtggctgtctgacggaagagcgcgtgctgcacctccctagtatggtgggcgaggattgtgtggatgaggaagaccagccgcgagtggcggcacagcttgttctgagcgaactgcaccgagtccagtcgctggtgaac